European Patent Application EP 4 212 180 A1, published July 19, 2023. Title: MODIFIED THERAPEUTIC AGENTS, STAPLED PEPTIDE LIPID CONJUGATES, AND COMPOSITIONS THEREOF. Applicant: THE SCRIPPS RESEARCH INSTITUTE. Application US PCT/US2014/070977, filed December 17, 2014. The sequence listing filed with the application follows.

SEQUENCE LISTING (54 sequences)

SEQ ID NO: 1 - protein, 37 aa, Homo sapiens
HSQGTFTSDYSKYLDSRRAQDFVQWLMNTKRNRNNIA

SEQ ID NO: 2 - protein, 39 aa, Homo sapiens
HGEGTFTSDLSKQMEEEAVRLFIEWLKNGGPSSGAPPPS

SEQ ID NO: 3 - protein, 30 aa, Homo sapiens
HAEGTFTSDVSSYLEGQAAKEFIAWLVKGR

SEQ ID NO: 4 - protein, 29 aa, Homo sapiens
HSQGTFTSDYSKYLDSRRAQDFVQWLMNT

SEQ ID NO: 5 - protein, 33 aa, Homo sapiens
HADGSFSDEMNTILDNLAARDFINWLIQTKITD

SEQ ID NO: 6 - protein, 42 aa, Homo sapiens
YAEGTFISDYSIAMDKIHQQDFVNWLLAQKGKKNDWKHNITQ

SEQ ID NO: 7 - protein, 38 aa, synthetic construct
  REGION 1..38: note = Description of Artificial Sequence: Syntheticpolypeptide
  SITE 2: note = D-Serine
HSQGTFTSDYSKYLDSRRAQDFVQWLMNTKRNRNNIAC

SEQ ID NO: 8 - protein, 37 aa, synthetic construct
  REGION 1..37: note = Description of Artificial Sequence: Syntheticpolypeptide
  SITE 2: note = D-Serine
HSQGTFTSDYSKYLDERAACEFICWLMNTKRNRNNIA

SEQ ID NO: 9 - protein, 37 aa, synthetic construct
  REGION 1..37: note = Description of Artificial Sequence: Syntheticpolypeptide
  SITE 2: note = D-Serine
HSQGTFTSDYSKCLDERAVRLFICWLMNTKRNRNNIA

SEQ ID NO: 10 - protein, 37 aa, synthetic construct
  REGION 1..37: note = Description of Artificial Sequence: Syntheticpolypeptide
  SITE 2: note = D-Serine
HSQGTFTSDCSKYLDERAVRLFICWLMNTKRNRNNIA

SEQ ID NO: 11 - protein, 37 aa, synthetic construct
  REGION 1..37: note = Description of Artificial Sequence: Syntheticpolypeptide
  SITE 2: note = D-Serine
HSQGTFTSCYSKCLDECAVRLFICWLMNTKRNRNNIA

SEQ ID NO: 12 - protein, 37 aa, synthetic construct
  REGION 1..37: note = Description of Artificial Sequence: Syntheticpolypeptide
  SITE 2: note = D-Serine
HSQGTFTSCYSKCLDERAVRLFICWLMNTKRNRNNIA

SEQ ID NO: 13 - protein, 39 aa, synthetic construct
  REGION 1..39: note = Description of Artificial Sequence: Syntheticpolypeptide
HGEGTFTSDLSKQMEECAVRLFICWLKNGGPSSGAPPPS

SEQ ID NO: 14 - protein, 40 aa, synthetic construct
  REGION 1..40: note = Description of Artificial Sequence: Syntheticpolypeptide
HGEGTFTSDLSKQMEECAVRLFICWLKNGGPSSGAPPPSC

SEQ ID NO: 15 - protein, 39 aa, synthetic construct
  REGION 1..39: note = Description of Artificial Sequence: Syntheticpolypeptide
HGEGTFTSDLSKQMEEEAVCLFICWLKNGGPSSGAPPPS

SEQ ID NO: 16 - protein, 39 aa, synthetic construct
  REGION 1..39: note = Description of Artificial Sequence: Syntheticpolypeptide
HGEGTFTSDLSKCMEEEAVRLFICWLKNGGPSSGAPPPS

SEQ ID NO: 17 - protein, 39 aa, synthetic construct
  REGION 1..39: note = Description of Artificial Sequence: Syntheticpolypeptide
HGEGTFTSDCSKQMEEEAVRLFICWLKNGGPSSGAPPPS

SEQ ID NO: 18 - protein, 39 aa, synthetic construct
  REGION 1..39: note = Description of Artificial Sequence: Syntheticpolypeptide
HGEGTFTSCLSKQMEEEAVRLFICWLKNGGPSSGAPPPS

SEQ ID NO: 19 - protein, 39 aa, synthetic construct
  REGION 1..39: note = Description of Artificial Sequence: Syntheticpolypeptide
HGEGTFTSCLSKCMEEEAVRLFICWLKNGGPSSGAPPPS

SEQ ID NO: 20 - protein, 29 aa, synthetic construct
  REGION 1..29: note = Description of Artificial Sequence: Syntheticpeptide
  SITE 2: note = D-Serine
HSQGTFTSDYSKYLDSKAAHDFVCWLLRA

SEQ ID NO: 21 - protein, 29 aa, synthetic construct
  REGION 1..29: note = Description of Artificial Sequence: Syntheticpeptide
HSQGTFTSDYSKYLDSCAAHDFVCWLLRA

SEQ ID NO: 22 - protein, 29 aa, synthetic construct
  REGION 1..29: note = Description of Artificial Sequence: Syntheticpeptide
  SITE 2: note = D-Serine
HSQGTFTSDYSKCLDSKAAHDFVCWLLRA

SEQ ID NO: 23 - protein, 29 aa, synthetic construct
  REGION 1..29: note = Description of Artificial Sequence: Syntheticpeptide
  SITE 2: note = D-Serine
HSQGTFTSCYSKYLDSKAAHDFVCWLLRA

SEQ ID NO: 24 - protein, 29 aa, synthetic construct
  REGION 1..29: note = Description of Artificial Sequence: Syntheticpeptide
  SITE 2: note = D-Serine
HSQGTFTSCYSKCLDSCAAHDFVCWLLRA

SEQ ID NO: 25 - protein, 40 aa, synthetic construct
  REGION 1..40: note = Description of Artificial Sequence: Syntheticpolypeptide
  VARIANT 2: note = X can be any amino acid
YXEGTFTSDYSIYLDKQAACEFVCWLLAGGPSSGAPPPSK

SEQ ID NO: 26 - protein, 40 aa, synthetic construct
  REGION 1..40: note = Description of Artificial Sequence: Syntheticpolypeptide
  VARIANT 2: note = X can be any amino acid
  VARIANT 20: note = X can be any amino acid
YXEGTFTSDYSIYLDKCAAXEFVCWLLAGGPSSGAPPPSK

SEQ ID NO: 27 - protein, 40 aa, synthetic construct
  REGION 1..40: note = Description of Artificial Sequence: Syntheticpolypeptide
  VARIANT 2: note = X can be any amino acid
  VARIANT 20: note = X can be any amino acid
YXEGTFTSDYSICLDKQAAXEFVCWLLAGGPSSGAPPPSK

SEQ ID NO: 28 - protein, 40 aa, synthetic construct
  REGION 1..40: note = Description of Artificial Sequence: Syntheticpolypeptide
  VARIANT 2: note = X can be any amino acid
  VARIANT 20: note = X can be any amino acid
YXEGTFTSDCSIYLDKQAAXEFVCWLLAGGPSSGAPPPSK

SEQ ID NO: 29 - protein, 40 aa, synthetic construct
  REGION 1..40: note = Description of Artificial Sequence: Syntheticpolypeptide
  VARIANT 2: note = X can be any amino acid
  VARIANT 20: note = X can be any amino acid
YXEGTFTSCYSICLDKQAAXEFVCWLLAGGPSSGAPPPSK

SEQ ID NO: 30 - protein, 39 aa, synthetic construct; identical to SEQ ID NO: 13
  REGION 1..39: note = Description of Artificial Sequence: Syntheticpolypeptide

SEQ ID NO: 31 - protein, 39 aa, synthetic construct; identical to SEQ ID NO: 16
  REGION 1..39: note = Description of Artificial Sequence: Syntheticpolypeptide

SEQ ID NO: 32 - protein, 39 aa, synthetic construct; identical to SEQ ID NO: 17
  REGION 1..39: note = Description of Artificial Sequence: Syntheticpolypeptide

SEQ ID NO: 33 - protein, 37 aa, synthetic construct
  REGION 1..37: note = Description of Artificial Sequence: Syntheticpolypeptide
  SITE 2: note = D-Serine
HSQGTFTSDYSKYLDSCRAQDFVCWLMNTKRNRNNIA

SEQ ID NO: 34 - protein, 37 aa, synthetic construct
  REGION 1..37: note = Description of Artificial Sequence: Syntheticpolypeptide
  SITE 2: note = D-Serine
HSQGTFTSDYSKYLDECAAKEFICWLMNTKRNRNNIA

SEQ ID NO: 35 - protein, 29 aa, synthetic construct
  REGION 1..29: note = Description of Artificial Sequence: Syntheticpeptide
  SITE 2: note = D-Serine
HSQGTFTSDYSKYLDSCAAHDFVCWLLRA

SEQ ID NO: 36 - protein, 29 aa, synthetic construct
  REGION 1..29: note = Description of Artificial Sequence: Syntheticpeptide
  SITE 2: note = D-Serine
HSQGTFTSDYSKYLDECAAKEFICWLLRA

SEQ ID NO: 37 - protein, 39 aa, synthetic construct
  REGION 1..39: note = Description of Artificial Sequence: Syntheticpolypeptide
  SITE 2: note = D-Serine
HSQGTFTSDYSKYLDECAAKEFICWLLRAGPSSGAPPPS

SEQ ID NO: 38 - protein, 39 aa, synthetic construct
  REGION 1..39: note = Description of Artificial Sequence: Syntheticpolypeptide
  SITE 2: note = D-Serine
HSQGTFTSDYSKYLDECAAKEFICWLLNGGPSSGAPPPS

SEQ ID NO: 39 - protein, 40 aa, synthetic construct
  REGION 1..40: note = Description of Artificial Sequence: Syntheticpolypeptide
  SITE 2: note = D-Alanine
YAEGTFTSDYSIYLDKCAAKEFVCWLLAGGPSSGAPPPSK

SEQ ID NO: 40 - protein, 37 aa, synthetic construct
  REGION 1..37: note = Description of Artificial Sequence: Syntheticpolypeptide
  SITE 2: note = D-Alanine
YAEGTFISDYSKYLDECAAKEFICWLMNTKRNRNNIA

SEQ ID NO: 41 - protein, 39 aa, synthetic construct
  REGION 1..39: note = Description of Artificial Sequence: Syntheticpolypeptide
  MOD_RES 2: note = Aib
HXQGTFTSDKSKYLDECAAQDFVCWLLDGGPSSGAPPPS

SEQ ID NO: 42 - protein, 33 aa, synthetic construct
  REGION 1..33: note = Description of Artificial Sequence: Syntheticpolypeptide
HGDGSFSDEMNTILDNCAARDFICWLIQTKITD

SEQ ID NO: 43 - protein, 33 aa, synthetic construct
  REGION 1..33: note = Description of Artificial Sequence: Syntheticpolypeptide
HGDGSFSDELLTILDLCAARDFICWLIQTKITD

SEQ ID NO: 44 - protein, 33 aa, synthetic construct
  REGION 1..33: note = Description of Artificial Sequence: Syntheticpolypeptide
HGDGSFSDEMNTILDCLAARDFICWLIQTKITD

SEQ ID NO: 45 - protein, 33 aa, synthetic construct
  REGION 1..33: note = Description of Artificial Sequence: Syntheticpolypeptide
HGDGSFSCEMNTILCALAARDFINWLIQTKITD

SEQ ID NO: 46 - protein, 33 aa, synthetic construct
  REGION 1..33: note = Description of Artificial Sequence: Syntheticpolypeptide
HGDGSFSDEMNTILDALAARCFINWLICTKITD

SEQ ID NO: 47 - protein, 33 aa, synthetic construct
  REGION 1..33: note = Description of Artificial Sequence: Syntheticpolypeptide
HGDGSFSDCMNTILDCLAARDFINWLIQTKITD

SEQ ID NO: 48 - protein, 33 aa, synthetic construct
  REGION 1..33: note = Description of Artificial Sequence: Syntheticpolypeptide
HGDGSFSDEMCTILDNLCARDFINWLIQTKITD

SEQ ID NO: 49 - protein, 42 aa, synthetic construct
  REGION 1..42: note = Description of Artificial Sequence: Syntheticpolypeptide
HGDGSFSDEMNTILDNCAARDFICWLIQTKITDPSSGAPPPS

SEQ ID NO: 50 - protein, 42 aa, synthetic construct
  REGION 1..42: note = Description of Artificial Sequence: Syntheticpolypeptide
HGDGSFSDCMNTILDCLAARDFINWLIQTKITDPSSGAPPPS

SEQ ID NO: 51 - protein, 42 aa, synthetic construct
  REGION 1..42: note = Description of Artificial Sequence: Syntheticpolypeptide
HGDGSFSDEMCTILDNLCARDFINWLIQTKITDPSSGAPPPS

SEQ ID NO: 52 - protein, 30 aa, synthetic construct
  REGION 1..30: note = Description of Artificial Sequence: Syntheticpolypeptide
HGEGTFTSDVSSYLEGCAAKEFICWLVKGR

SEQ ID NO: 53 - protein, 30 aa, synthetic construct
  REGION 1..30: note = Description of Artificial Sequence: Syntheticpolypeptide
  MOD_RES 2: note = Aib
HXEGTFTSDVSSYLEGCAAKEFICWLVKGR

SEQ ID NO: 54 - protein, 38 aa, synthetic construct
  REGION 1..38: note = Description of Artificial Sequence: Syntheticpolypeptide
  SITE 2: note = D-Serine
HSQGTFTSDYSKYLDECAAKEFICWLMNTKRNRNNIAC